European Patent Application EP 4 792 824 A1, published August 19, 2026. Title: Peptide hydrogels and their use for skeletal muscle regeneration as stimulators of myoblast migration and fusion. Applicant: University of Warsaw. Application PL -, filed January 16, 2025. The sequence listing filed with the application follows.

SEQUENCE LISTING (18 sequences)

SEQ ID NO: 1 - protein, 28 aa, synthetic construct
  MOD_RES <1: note = ACETYLATION
  MOD_RES >28: note = AMIDATION
RADARADARADARADAVLGLKPVSLSYR

SEQ ID NO: 2 - protein, 31 aa, synthetic construct
  MOD_RES <1: note = ACETYLATION
  MOD_RES >31: note = AMIDATION
RADARADARADARADAVLGLVARLKNNNRQV

SEQ ID NO: 3 - protein, 31 aa, synthetic construct
  MOD_RES <1: note = ACETYLATION
  MOD_RES >31: note = AMIDATION
RADARADARADARADAVLGLITLQEIIKTLN

SEQ ID NO: 4 - protein, 35 aa, synthetic construct
  MOD_RES <1: note = ACETYLATION
  MOD_RES >35: note = AMIDATION
RADARADARADARADAVLGLQLIRFLKRLDRNLWG

SEQ ID NO: 5 - protein, 31 aa, synthetic construct
  MOD_RES <1: note = ACETYLATION
  MOD_RES >31: note = AMIDATION
RADARADARADARADAGGGPAGLKPVSLSYR

SEQ ID NO: 6 - protein, 34 aa, synthetic construct
  MOD_RES <1: note = ACETYLATION
  MOD_RES >34: note = AMIDATION
RADARADARADARADAGGGPAGLVARLKNNNRQV

SEQ ID NO: 7 - protein, 34 aa, synthetic construct
  MOD_RES <1: note = ACETYLATION
  MOD_RES >34: note = AMIDATION
RADARADARADARADAGGGPAGLITLQEIIKTLN

SEQ ID NO: 8 - protein, 38 aa, synthetic construct
  MOD_RES <1: note = ACETYLATION
  MOD_RES >38: note = AMIDATION
RADARADARADARADAGGGPAGLQLIRFLKRLDRNLWG

SEQ ID NO: 9 - protein, 16 aa, synthetic construct
  MOD_RES <1: note = ACETYLATION
  MOD_RES >16: note = AMIDATION
RADARADARADARADA

SEQ ID NO: 10 - protein, 20 aa, synthetic construct
  MOD_RES <1: note = ACETYLATION
  MOD_RES >20: note = AMIDATION
RADARADARADARADAVLGL

SEQ ID NO: 11 - protein, 23 aa, synthetic construct
  MOD_RES <1: note = ACETYLATION
RADARADARADARADAGGGPAGL

SEQ ID NO: 12 - protein, 23 aa, synthetic construct
  MOD_RES <1: note = ACETYLATION
  MOD_RES >23: note = AMIDATION
RADARADARADARADAVLGLRGD

SEQ ID NO: 13 - protein, 26 aa, synthetic construct
  MOD_RES <1: note = ACETYLATION
  MOD_RES 26: note = AMIDATION
RADARADARADARADAGGGPAGLRGD

SEQ ID NO: 14 - protein, 4 aa, synthetic construct
VLGL

SEQ ID NO: 15 - skipped

SEQ ID NO: 16 - protein, 4 aa, synthetic construct
PAGL

SEQ ID NO: 17 - skipped

SEQ ID NO: 18 - protein, 7 aa, synthetic construct
GGGPAGL